European Patent Application EP 4 538 290 A1, published April 16, 2025. Title: Fusion Protein Comprising Antibody Specifically Binding to TIGIT and Interleukin-15, and Uses thereof. Applicant: MediMabBio Inc. The sequence listing filed with the application follows.

SEQUENCE LISTING (125 sequences)

SEQ ID NO: 1 - protein, 6 aa, synthetic construct
  REGION 1..6: note = CDR-H1
SDYAWN

SEQ ID NO: 2 - protein, 10 aa, synthetic construct
  REGION 1..10: note = CDR-H1
GSTFTEYTMH

SEQ ID NO: 3 - protein, 10 aa, synthetic construct
  REGION 1..10: note = CDR-H1
GYSFTDYIMN

SEQ ID NO: 4 - protein, 16 aa, synthetic construct
  REGION 1..16: note = CDR-H2
YISYSGSARYNPSLKS

SEQ ID NO: 5 - protein, 17 aa, synthetic construct
  REGION 1..17: note = CDR-H2
GLNPNNGGTSYNQRFKD

SEQ ID NO: 6 - protein, 17 aa, synthetic construct
  REGION 1..17: note = CDR-H2
LSIPYNGGTSYNQKFEG

SEQ ID NO: 7 - protein, 9 aa, synthetic construct
  REGION 1..9: note = CDR-H3
KGYPAYFAY

SEQ ID NO: 8 - protein, 10 aa, synthetic construct
  REGION 1..10: note = CDR-H3
GTYYDYSFAY

SEQ ID NO: 9 - protein, 10 aa, synthetic construct
  REGION 1..10: note = CDR-H3
GIKGYFAMDY

SEQ ID NO: 10 - protein, 11 aa, synthetic construct
  REGION 1..11: note = CDR-L1
  VARIANT 1: note = Xaa is Lys(K) or Arg(R)
XASQDVSTAVA

SEQ ID NO: 11 - protein, 11 aa, synthetic construct
  REGION 1..11: note = CDR-L1
KASQDVSTAVA

SEQ ID NO: 12 - protein, 11 aa, synthetic construct
  REGION 1..11: note = CDR-L1
RASQDVSTAVA

SEQ ID NO: 13 - protein, 11 aa, synthetic construct
  REGION 1..11: note = CDR-L1
KASHYVSTAVA

SEQ ID NO: 14 - protein, 16 aa, synthetic construct
  REGION 1..16: note = CDR-L1
RSSQSLVNSFGKTYLS

SEQ ID NO: 15 - protein, 7 aa, synthetic construct
  REGION 1..7: note = CDR-L2
SASYRYT

SEQ ID NO: 16 - protein, 7 aa, synthetic construct
  REGION 1..7: note = CDR-L2
SPSYRYT

SEQ ID NO: 17 - protein, 7 aa, synthetic construct
  REGION 1..7: note = CDR-L2
GVSNRFS

SEQ ID NO: 18 - protein, 9 aa, synthetic construct
  REGION 1..9: note = CDR-L3
QHHYSTPYT

SEQ ID NO: 19 - protein, 9 aa, synthetic construct
  REGION 1..9: note = CDR-L3
HQHYSTPWT

SEQ ID NO: 20 - protein, 9 aa, synthetic construct
  REGION 1..9: note = CDR-L3
LQGTHQPWT

SEQ ID NO: 21 - protein, 118 aa, synthetic construct
  REGION 1..118: note = heavy chain variable region of anti-TIGIT antibody
DVQLQESGPGLVKPSQSLSLTCTVTGYSITSDYAWNWIRQFPGNKLEWMGYISYSGSARYNPSLKSRISITRDTSMNQFFLQLNSVTAEDTATYYCARKGYPAYFAYWGQGTLVTVSS

SEQ ID NO: 22 - protein, 118 aa, synthetic construct
  REGION 1..118: note = heavy chain variable region of anti-TIGIT antibody
DVQLQESGPGLVKPSQTLSLTCTVTGYSITSDYAWNWIRQPPGKGLEWMGYISYSGSARYNPSLKSRITISRDTSMNQFSLKLNSVTAEDTATYYCARKGYPAYFAYWGQGTLVTVSS

SEQ ID NO: 23 - protein, 118 aa, synthetic construct
  REGION 1..118: note = heavy chain variable region of anti-TIGIT antibody
DVQLQESGPGLVKPSQTLSLTCTVTGYSITSDYAWNWIRQPPGKGLEWMGYISYSGSARYNPSLKSRITISRDTSKNQFSLKLSSVTAEDTATYYCARKGYPAYFAYWGQGTLVTVSS

SEQ ID NO: 24 - protein, 118 aa, synthetic construct
  REGION 1..118: note = heavy chain variable region of anti-TIGIT antibody
QVQLQESGPGLVKPSQTLSLTCTVTGYSITSDYAWNWIRQPPGKGLEWMGYISYSGSARYNPSLKSRVTISRDTSKNQFSLKLSSVTAEDTATYYCARKGYPAYFAYWGQGTLVTVSS

SEQ ID NO: 25 - protein, 118 aa, synthetic construct
  REGION 1..118: note = heavy chain variable region of anti-TIGIT antibody
QVQLQESGPGLVKPSQTLSLTCTVTGYSITSDYAWNWIRQPPGKGLEWMGYISYSGSARYNPSLKSRVTISRDTSKNQFSLKLSSVTAADTAVYYCARKGYPAYFAYWGQGTLVTVSS

SEQ ID NO: 26 - protein, 118 aa, synthetic construct
  REGION 1..118: note = heavy chain variable region of anti-TIGIT antibody
QVQLQESGPGLVKPSQTLSLTCTVTGYSITSDYAWNWIRQPPGKGLEWMGYISYSGSARYNPSLKSRVTISVDTSKNQFSLKLSSVTAADTAVYYCARKGYPAYFAYWGQGTLVTVSS

SEQ ID NO: 27 - protein, 119 aa, synthetic construct
  REGION 1..119: note = heavy chain variable region of anti-TIGIT antibody
EVQLQQSGPELVKPGASVKISCKTSGSTFTEYTMHWVKQSHGKSLEWIGGLNPNNGGTSYNQRFKDRATLTVDKSSSTAYMELRSLTSEDSAVYYCTRGTYYDYSFAYWGQGTLVTVSA

SEQ ID NO: 28 - protein, 119 aa, synthetic construct
  REGION 1..119: note = heavy chain variable region of anti-TIGIT antibody
EVQLQQSGPELVKPGASMKISCKASGYSFTDYIMNWVKQSHGKNLEWIGLSIPYNGGTSYNQKFEGKATLTVDKSSSTAYMELLSLTSEDSAVYYCARGIKGYFAMDYWGQGTSVTVSS

SEQ ID NO: 29 - protein, 107 aa, synthetic construct
  REGION 1..107: note = light chain variable region of anti-TIGIT antibody
DIVMTQSHKFMSTSVGDRVSISCKASQDVSTAVAWYQQKPGQSPELLIYSASYRYTGVPDRFTGSGSGTDFTFTISSVQAEDLAVYYCQHHYSTPYTFGGGTKLEMK

SEQ ID NO: 30 - protein, 107 aa, synthetic construct
  REGION 1..107: note = light chain variable region of anti-TIGIT antibody
DIVMTQSHSFLSASVGDRVSITCKASQDVSTAVAWYQQKPGQAPELLIYSASYRYTGVPDRFTGSGSGTDFTLTISSLQAEDVAVYYCQHHYSTPYTFGQGTKLEMK

SEQ ID NO: 31 - protein, 107 aa, synthetic construct
  REGION 1..107: note = light chain variable region of anti-TIGIT antibody
DIVMTQSPSSLSASVGDRVSITCKASQDVSTAVAWYQQKPGQAPRLLIYSASYRYTGVPDRFTGSGSGTDFTLTISSLQAEDVAVYYCQHHYSTPYTFGQGTKLEIK

SEQ ID NO: 32 - protein, 107 aa, synthetic construct
  REGION 1..107: note = light chain variable region of anti-TIGIT antibody
DIQMTQSPSSLSASVGDRVSITCKASQDVSTAVAWYQQKPGQAPRLLIYSASYRYTGVPDRFSGSGSGTDFTLTISSLQAEDVAVYYCQHHYSTPYTFGQGTKLEIK

SEQ ID NO: 33 - protein, 107 aa, synthetic construct
  REGION 1..107: note = light chain variable region of anti-TIGIT antibody
DIQMTQSPSSLSASVGDRVTITCRASQDVSTAVAWYQQKPGQAPRLLIYSASYRYTGVPDRFSGSGSGTDFTLTISSLQAEDVAVYYCQHHYSTPYTFGQGTKLEIK

SEQ ID NO: 34 - protein, 107 aa, synthetic construct
  REGION 1..107: note = light chain variable region of anti-TIGIT antibody
DIQMTQSPSSLSASVGDRVSITCKASQDVSTAVAWYQQKPGQAPRLLIYSASYRYTGVPDRFSGSGSGTDFTLTISSLQPEDFATYYCQHHYSTPYTFGQGTKLEIK

SEQ ID NO: 35 - protein, 107 aa, synthetic construct
  REGION 1..107: note = light chain variable region of anti-TIGIT antibody
DIVMTQSHKFMSTSVGDRVSITCKASHYVSTAVAWYQQKPGQSPKLLIYSPSYRYTGVPDRFTGSGSGTDFTFTISSVQAEDLAVYYCHQHYSTPWTFGGGTKLEIK

SEQ ID NO: 36 - protein, 112 aa, synthetic construct
  REGION 1..112: note = light chain variable region of anti-TIGIT antibody
DVVVTQTPLSLPVSFGDQVSISCRSSQSLVNSFGKTYLSWFLHKPGQSPQLIMYGVSNRFSGVPDRFSGSGSGTDFTLKISTIKPEDLGMYYCLQGTHQPWTFGGGTKLEIK

SEQ ID NO: 37 - protein, 20 aa, synthetic construct
  REGION 1..20: note = aa 51-70 of hTIGIT
TAQVTQVNWEQQDQLLAICN

SEQ ID NO: 38 - protein, 114 aa, synthetic construct
  REGION 1..114: note = IL-15
NWVNVISDLKKIEDLIQSMHIDATLYTESDVHPSCKVTAMKCFLLELQVISLESGDASIHDTVENLIILANNSLSSNGNVTESGCKECEELEEKNIKEFLQSFVHIVQMFINTS

SEQ ID NO: 39 - protein, 15 aa, synthetic construct
  REGION 1..15: note = peptide linker (flexible)
GGGGSGGGGSGGGGS

SEQ ID NO: 40 - protein, 15 aa, synthetic construct
  REGION 1..15: note = peptide linker (rigid)
EAAAKEAAAKEAAAK

SEQ ID NO: 41 - protein, 330 aa, synthetic construct
  REGION 1..330: note = heavy chain constant region
ASTKGPSVFPLAPSSKSTSGGTAALGCLVKDYFPEPVTVSWNSGALTSGVHTFPAVLQSSGLYSLSSVVTVPSSSLGTQTYICNVNHKPSNTKVDKRVEPKSCDKTHTCPPCPAPELLGGPSVFLFPPKPKDTLMISRTPEVTCVVVDVSHEDPEVKFNWYVDGVEVHNAKTKPREEQYNSTYRVVSVLTVLHQDWLNGKEYKCKVSNKALPAPIEKTISKAKGQPREPQVYTLPPSREEMTKNQVSLTCLVKGFYPSDIAVEWESNGQPENNYKTTPPVLDSDGSFFLYSKLTVDKSRWQQGNVFSCSVMHEALHNHYTQKSLSLSPGK

SEQ ID NO: 42 - protein, 448 aa, synthetic construct
  REGION 1..448: note = heavy chain (7A6)
QVQLQESGPGLVKPSQTLSLTCTVTGYSITSDYAWNWIRQPPGKGLEWMGYISYSGSARYNPSLKSRVTISRDTSKNQFSLKLSSVTAEDTATYYCARKGYPAYFAYWGQGTLVTVSSASTKGPSVFPLAPSSKSTSGGTAALGCLVKDYFPEPVTVSWNSGALTSGVHTFPAVLQSSGLYSLSSVVTVPSSSLGTQTYICNVNHKPSNTKVDKRVEPKSCDKTHTCPPCPAPELLGGPSVFLFPPKPKDTLMISRTPEVTCVVVDVSHEDPEVKFNWYVDGVEVHNAKTKPREEQYNSTYRVVSVLTVLHQDWLNGKEYKCKVSNKALPAPIEKTISKAKGQPREPQVYTLPPSREEMTKNQVSLTCLVKGFYPSDIAVEWESNGQPENNYKTTPPVLDSDGSFFLYSKLTVDKSRWQQGNVFSCSVMHEALHNHYTQKSLSLSPGK

SEQ ID NO: 43 - protein, 107 aa, synthetic construct [sequence omitted]

SEQ ID NO: 44 - protein, 214 aa, synthetic construct
  REGION 1..214: note = light chain (7A6)
DIQMTQSPSSLSASVGDRVSITCKASQDVSTAVAWYQQKPGQAPRLLIYSASYRYTGVPDRFSGSGSGTDFTLTISSLQPEDFATYYCQHHYSTPYTFGQGTKLEIKRTVAAPSVFIFPPSDEQLKSGTASVVCLLNNFYPREAKVQWKVDNALQSGNSQESVTEQDSKDSTYSLSSTLTLSKADYEKHKVYACEVTHQGLSSPVTKSFNRGEC

SEQ ID NO: 45 - protein, 343 aa, synthetic construct
  REGION 1..343: note = light chian strand (7A615 TL-1)
DIQMTQSPSSLSASVGDRVSITCKASQDVSTAVAWYQQKPGQAPRLLIYSASYRYTGVPDRFSGSGSGTDFTLTISSLQPEDFATYYCQHHYSTPYTFGQGTKLEIKRTVAAPSVFIFPPSDEQLKSGTASVVCLLNNFYPREAKVQWKVDNALQSGNSQESVTEQDSKDSTYSLSSTLTLSKADYEKHKVYACEVTHQGLSSPVTKSFNRGECGGGGSGGGGSGGGGSNWVNVISDLKKIEDLIQSMHIDATLYTESDVHPSCKVTAMKCFLLELQVISLESGDASIHDTVENLIILANNSLSSNGNVTESGCKECEELEEKNIKEFLQSFVHIVQMFINTS

SEQ ID NO: 46 - protein, 343 aa, synthetic construct
  REGION 1..343: note = light chian strand (7A615 TL-2)
DIQMTQSPSSLSASVGDRVSITCKASQDVSTAVAWYQQKPGQAPRLLIYSASYRYTGVPDRFSGSGSGTDFTLTISSLQPEDFATYYCQHHYSTPYTFGQGTKLEIKRTVAAPSVFIFPPSDEQLKSGTASVVCLLNNFYPREAKVQWKVDNALQSGNSQESVTEQDSKDSTYSLSSTLTLSKADYEKHKVYACEVTHQGLSSPVTKSFNRGECEAAAKEAAAKEAAAKNWVNVISDLKKIEDLIQSMHIDATLYTESDVHPSCKVTAMKCFLLELQVISLESGDASIHDTVENLIILANNSLSSNGNVTESGCKECEELEEKNIKEFLQSFVHIVQMFINTS

SEQ ID NO: 47 - protein, 577 aa, synthetic construct
  REGION 1..577: note = heavy chian strand (7A615 TL-3)
QVQLQESGPGLVKPSQTLSLTCTVTGYSITSDYAWNWIRQPPGKGLEWMGYISYSGSARYNPSLKSRVTISRDTSKNQFSLKLSSVTAEDTATYYCARKGYPAYFAYWGQGTLVTVSSASTKGPSVFPLAPSSKSTSGGTAALGCLVKDYFPEPVTVSWNSGALTSGVHTFPAVLQSSGLYSLSSVVTVPSSSLGTQTYICNVNHKPSNTKVDKRVEPKSCDKTHTCPPCPAPELLGGPSVFLFPPKPKDTLMISRTPEVTCVVVDVSHEDPEVKFNWYVDGVEVHNAKTKPREEQYNSTYRVVSVLTVLHQDWLNGKEYKCKVSNKALPAPIEKTISKAKGQPREPQVYTLPPSREEMTKNQVSLTCLVKGFYPSDIAVEWESNGQPENNYKTTPPVLDSDGSFFLYSKLTVDKSRWQQGNVFSCSVMHEALHNHYTQKSLSLSPGKGGGGSGGGGSGGGGSNWVNVISDLKKIEDLIQSMHIDATLYTESDVHPSCKVTAMKCFLLELQVISLESGDASIHDTVENLIILANNSLSSNGNVTESGCKECEELEEKNIKEFLQSFVHIVQMFINTS

SEQ ID NO: 48 - protein, 577 aa, synthetic construct
  REGION 1..577: note = heavy chian strand (7A615 TL-4)
QVQLQESGPGLVKPSQTLSLTCTVTGYSITSDYAWNWIRQPPGKGLEWMGYISYSGSARYNPSLKSRVTISRDTSKNQFSLKLSSVTAEDTATYYCARKGYPAYFAYWGQGTLVTVSSASTKGPSVFPLAPSSKSTSGGTAALGCLVKDYFPEPVTVSWNSGALTSGVHTFPAVLQSSGLYSLSSVVTVPSSSLGTQTYICNVNHKPSNTKVDKRVEPKSCDKTHTCPPCPAPELLGGPSVFLFPPKPKDTLMISRTPEVTCVVVDVSHEDPEVKFNWYVDGVEVHNAKTKPREEQYNSTYRVVSVLTVLHQDWLNGKEYKCKVSNKALPAPIEKTISKAKGQPREPQVYTLPPSREEMTKNQVSLTCLVKGFYPSDIAVEWESNGQPENNYKTTPPVLDSDGSFFLYSKLTVDKSRWQQGNVFSCSVMHEALHNHYTQKSLSLSPGKEAAAKEAAAKEAAAKNWVNVISDLKKIEDLIQSMHIDATLYTESDVHPSCKVTAMKCFLLELQVISLESGDASIHDTVENLIILANNSLSSNGNVTESGCKECEELEEKNIKEFLQSFVHIVQMFINTS

SEQ ID NO: 49 - protein, 562 aa, synthetic construct
  REGION 1..562: note = heavy chian strand (7A615 TL-5)
QVQLQESGPGLVKPSQTLSLTCTVTGYSITSDYAWNWIRQPPGKGLEWMGYISYSGSARYNPSLKSRVTISRDTSKNQFSLKLSSVTAEDTATYYCARKGYPAYFAYWGQGTLVTVSSASTKGPSVFPLAPSSKSTSGGTAALGCLVKDYFPEPVTVSWNSGALTSGVHTFPAVLQSSGLYSLSSVVTVPSSSLGTQTYICNVNHKPSNTKVDKRVEPKSCDKTHTCPPCPAPELLGGPSVFLFPPKPKDTLMISRTPEVTCVVVDVSHEDPEVKFNWYVDGVEVHNAKTKPREEQYNSTYRVVSVLTVLHQDWLNGKEYKCKVSNKALPAPIEKTISKAKGQPREPQVYTLPPSREEMTKNQVSLTCLVKGFYPSDIAVEWESNGQPENNYKTTPPVLDSDGSFFLYSKLTVDKSRWQQGNVFSCSVMHEALHNHYTQKSLSLSPGKNWVNVISDLKKIEDLIQSMHIDATLYTESDVHPSCKVTAMKCFLLELQVISLESGDASIHDTVENLIILANNSLSSNGNVTESGCKECEELEEKNIKEFLQSFVHIVQMFINTS

SEQ ID NO: 50 - protein, 449 aa, synthetic construct
  REGION 1..449: note = heavy chain (2B7)
EVQLQQSGPELVKPGASVKISCKTSGSTFTEYTMHWVKQSHGKSLEWIGGLNPNNGGTSYNQRFKDRATLTVDKSSSTAYMELRSLTSEDSAVYYCTRGTYYDYSFAYWGQGTLVTVSAASTKGPSVFPLAPSSKSTSGGTAALGCLVKDYFPEPVTVSWNSGALTSGVHTFPAVLQSSGLYSLSSVVTVPSSSLGTQTYICNVNHKPSNTKVDKRVEPKSCDKTHTCPPCPAPELLGGPSVFLFPPKPKDTLMISRTPEVTCVVVDVSHEDPEVKFNWYVDGVEVHNAKTKPREEQYNSTYRVVSVLTVLHQDWLNGKEYKCKVSNKALPAPIEKTISKAKGQPREPQVYTLPPSREEMTKNQVSLTCLVKGFYPSDIAVEWESNGQPENNYKTTPPVLDSDGSFFLYSKLTVDKSRWQQGNVFSCSVMHEALHNHYTQKSLSLSPGK

SEQ ID NO: 51 - protein, 214 aa, synthetic construct
  REGION 1..214: note = light chain (2B7)
DIVMTQSHKFMSTSVGDRVSITCKASHYVSTAVAWYQQKPGQSPKLLIYSPSYRYTGVPDRFTGSGSGTDFTFTISSVQAEDLAVYYCHQHYSTPWTFGGGTKLEIKRTVAAPSVFIFPPSDEQLKSGTASVVCLLNNFYPREAKVQWKVDNALQSGNSQESVTEQDSKDSTYSLSSTLTLSKADYEKHKVYACEVTHQGLSSPVTKSFNRGEC

SEQ ID NO: 52 - protein, 343 aa, synthetic construct
  REGION 1..343: note = light chian strand (2B715 TL-1)
DIVMTQSHKFMSTSVGDRVSITCKASHYVSTAVAWYQQKPGQSPKLLIYSPSYRYTGVPDRFTGSGSGTDFTFTISSVQAEDLAVYYCHQHYSTPWTFGGGTKLEIKRTVAAPSVFIFPPSDEQLKSGTASVVCLLNNFYPREAKVQWKVDNALQSGNSQESVTEQDSKDSTYSLSSTLTLSKADYEKHKVYACEVTHQGLSSPVTKSFNRGECGGGGSGGGGSGGGGSNWVNVISDLKKIEDLIQSMHIDATLYTESDVHPSCKVTAMKCFLLELQVISLESGDASIHDTVENLIILANNSLSSNGNVTESGCKECEELEEKNIKEFLQSFVHIVQMFINTS

SEQ ID NO: 53 - protein, 343 aa, synthetic construct
  REGION 1..343: note = light chian strand (2B715 TL-2)
DIVMTQSHKFMSTSVGDRVSITCKASHYVSTAVAWYQQKPGQSPKLLIYSPSYRYTGVPDRFTGSGSGTDFTFTISSVQAEDLAVYYCHQHYSTPWTFGGGTKLEIKRTVAAPSVFIFPPSDEQLKSGTASVVCLLNNFYPREAKVQWKVDNALQSGNSQESVTEQDSKDSTYSLSSTLTLSKADYEKHKVYACEVTHQGLSSPVTKSFNRGECEAAAKEAAAKEAAAKNWVNVISDLKKIEDLIQSMHIDATLYTESDVHPSCKVTAMKCFLLELQVISLESGDASIHDTVENLIILANNSLSSNGNVTESGCKECEELEEKNIKEFLQSFVHIVQMFINTS

SEQ ID NO: 54 - protein, 578 aa, synthetic construct
  REGION 1..578: note = heavy chian strand (2B715 TL-3)
EVQLQQSGPELVKPGASVKISCKTSGSTFTEYTMHWVKQSHGKSLEWIGGLNPNNGGTSYNQRFKDRATLTVDKSSSTAYMELRSLTSEDSAVYYCTRGTYYDYSFAYWGQGTLVTVSAASTKGPSVFPLAPSSKSTSGGTAALGCLVKDYFPEPVTVSWNSGALTSGVHTFPAVLQSSGLYSLSSVVTVPSSSLGTQTYICNVNHKPSNTKVDKRVEPKSCDKTHTCPPCPAPELLGGPSVFLFPPKPKDTLMISRTPEVTCVVVDVSHEDPEVKFNWYVDGVEVHNAKTKPREEQYNSTYRVVSVLTVLHQDWLNGKEYKCKVSNKALPAPIEKTISKAKGQPREPQVYTLPPSREEMTKNQVSLTCLVKGFYPSDIAVEWESNGQPENNYKTTPPVLDSDGSFFLYSKLTVDKSRWQQGNVFSCSVMHEALHNHYTQKSLSLSPGKGGGGSGGGGSGGGGSNWVNVISDLKKIEDLIQSMHIDATLYTESDVHPSCKVTAMKCFLLELQVISLESGDASIHDTVENLIILANNSLSSNGNVTESGCKECEELEEKNIKEFLQSFVHIVQMFINTS

SEQ ID NO: 55 - protein, 578 aa, synthetic construct
  REGION 1..578: note = heavy chian strand (2B715 TL-4)
EVQLQQSGPELVKPGASVKISCKTSGSTFTEYTMHWVKQSHGKSLEWIGGLNPNNGGTSYNQRFKDRATLTVDKSSSTAYMELRSLTSEDSAVYYCTRGTYYDYSFAYWGQGTLVTVSAASTKGPSVFPLAPSSKSTSGGTAALGCLVKDYFPEPVTVSWNSGALTSGVHTFPAVLQSSGLYSLSSVVTVPSSSLGTQTYICNVNHKPSNTKVDKRVEPKSCDKTHTCPPCPAPELLGGPSVFLFPPKPKDTLMISRTPEVTCVVVDVSHEDPEVKFNWYVDGVEVHNAKTKPREEQYNSTYRVVSVLTVLHQDWLNGKEYKCKVSNKALPAPIEKTISKAKGQPREPQVYTLPPSREEMTKNQVSLTCLVKGFYPSDIAVEWESNGQPENNYKTTPPVLDSDGSFFLYSKLTVDKSRWQQGNVFSCSVMHEALHNHYTQKSLSLSPGKEAAAKEAAAKEAAAKNWVNVISDLKKIEDLIQSMHIDATLYTESDVHPSCKVTAMKCFLLELQVISLESGDASIHDTVENLIILANNSLSSNGNVTESGCKECEELEEKNIKEFLQSFVHIVQMFINTS

SEQ ID NO: 56 - protein, 563 aa, synthetic construct
  REGION 1..563: note = heavy chian strand (2B715 TL-5)
EVQLQQSGPELVKPGASVKISCKTSGSTFTEYTMHWVKQSHGKSLEWIGGLNPNNGGTSYNQRFKDRATLTVDKSSSTAYMELRSLTSEDSAVYYCTRGTYYDYSFAYWGQGTLVTVSAASTKGPSVFPLAPSSKSTSGGTAALGCLVKDYFPEPVTVSWNSGALTSGVHTFPAVLQSSGLYSLSSVVTVPSSSLGTQTYICNVNHKPSNTKVDKRVEPKSCDKTHTCPPCPAPELLGGPSVFLFPPKPKDTLMISRTPEVTCVVVDVSHEDPEVKFNWYVDGVEVHNAKTKPREEQYNSTYRVVSVLTVLHQDWLNGKEYKCKVSNKALPAPIEKTISKAKGQPREPQVYTLPPSREEMTKNQVSLTCLVKGFYPSDIAVEWESNGQPENNYKTTPPVLDSDGSFFLYSKLTVDKSRWQQGNVFSCSVMHEALHNHYTQKSLSLSPGKNWVNVISDLKKIEDLIQSMHIDATLYTESDVHPSCKVTAMKCFLLELQVISLESGDASIHDTVENLIILANNSLSSNGNVTESGCKECEELEEKNIKEFLQSFVHIVQMFINTS

SEQ ID NO: 57 - protein, 449 aa, synthetic construct
  REGION 1..449: note = heavy chain (3F8)
EVQLQQSGPELVKPGASMKISCKASGYSFTDYIMNWVKQSHGKNLEWIGLSIPYNGGTSYNQKFEGKATLTVDKSSSTAYMELLSLTSEDSAVYYCARGIKGYFAMDYWGQGTSVTVSSASTKGPSVFPLAPSSKSTSGGTAALGCLVKDYFPEPVTVSWNSGALTSGVHTFPAVLQSSGLYSLSSVVTVPSSSLGTQTYICNVNHKPSNTKVDKRVEPKSCDKTHTCPPCPAPELLGGPSVFLFPPKPKDTLMISRTPEVTCVVVDVSHEDPEVKFNWYVDGVEVHNAKTKPREEQYNSTYRVVSVLTVLHQDWLNGKEYKCKVSNKALPAPIEKTISKAKGQPREPQVYTLPPSREEMTKNQVSLTCLVKGFYPSDIAVEWESNGQPENNYKTTPPVLDSDGSFFLYSKLTVDKSRWQQGNVFSCSVMHEALHNHYTQKSLSLSPGK

SEQ ID NO: 58 - protein, 219 aa, synthetic construct
  REGION 1..219: note = light chian (3F8)
DVVVTQTPLSLPVSFGDQVSISCRSSQSLVNSFGKTYLSWFLHKPGQSPQLIMYGVSNRFSGVPDRFSGSGSGTDFTLKISTIKPEDLGMYYCLQGTHQPWTFGGGTKLEIKRTVAAPSVFIFPPSDEQLKSGTASVVCLLNNFYPREAKVQWKVDNALQSGNSQESVTEQDSKDSTYSLSSTLTLSKADYEKHKVYACEVTHQGLSSPVTKSFNRGEC

SEQ ID NO: 59 - protein, 348 aa, synthetic construct
  REGION 1..348: note = light chian strand (3F815 TL-1)
DVVVTQTPLSLPVSFGDQVSISCRSSQSLVNSFGKTYLSWFLHKPGQSPQLIMYGVSNRFSGVPDRFSGSGSGTDFTLKISTIKPEDLGMYYCLQGTHQPWTFGGGTKLEIKRTVAAPSVFIFPPSDEQLKSGTASVVCLLNNFYPREAKVQWKVDNALQSGNSQESVTEQDSKDSTYSLSSTLTLSKADYEKHKVYACEVTHQGLSSPVTKSFNRGECGGGGSGGGGSGGGGSNWVNVISDLKKIEDLIQSMHIDATLYTESDVHPSCKVTAMKCFLLELQVISLESGDASIHDTVENLIILANNSLSSNGNVTESGCKECEELEEKNIKEFLQSFVHIVQMFINTS

SEQ ID NO: 60 - protein, 348 aa, synthetic construct
  REGION 1..348: note = light chian strand (3F815 TL-2)
DVVVTQTPLSLPVSFGDQVSISCRSSQSLVNSFGKTYLSWFLHKPGQSPQLIMYGVSNRFSGVPDRFSGSGSGTDFTLKISTIKPEDLGMYYCLQGTHQPWTFGGGTKLEIKRTVAAPSVFIFPPSDEQLKSGTASVVCLLNNFYPREAKVQWKVDNALQSGNSQESVTEQDSKDSTYSLSSTLTLSKADYEKHKVYACEVTHQGLSSPVTKSFNRGECEAAAKEAAAKEAAAKNWVNVISDLKKIEDLIQSMHIDATLYTESDVHPSCKVTAMKCFLLELQVISLESGDASIHDTVENLIILANNSLSSNGNVTESGCKECEELEEKNIKEFLQSFVHIVQMFINTS

SEQ ID NO: 61 - protein, 578 aa, synthetic construct
  REGION 1..578: note = heavy chian strand (3F815 TL-3)
EVQLQQSGPELVKPGASMKISCKASGYSFTDYIMNWVKQSHGKNLEWIGLSIPYNGGTSYNQKFEGKATLTVDKSSSTAYMELLSLTSEDSAVYYCARGIKGYFAMDYWGQGTSVTVSSASTKGPSVFPLAPSSKSTSGGTAALGCLVKDYFPEPVTVSWNSGALTSGVHTFPAVLQSSGLYSLSSVVTVPSSSLGTQTYICNVNHKPSNTKVDKRVEPKSCDKTHTCPPCPAPELLGGPSVFLFPPKPKDTLMISRTPEVTCVVVDVSHEDPEVKFNWYVDGVEVHNAKTKPREEQYNSTYRVVSVLTVLHQDWLNGKEYKCKVSNKALPAPIEKTISKAKGQPREPQVYTLPPSREEMTKNQVSLTCLVKGFYPSDIAVEWESNGQPENNYKTTPPVLDSDGSFFLYSKLTVDKSRWQQGNVFSCSVMHEALHNHYTQKSLSLSPGKGGGGSGGGGSGGGGSNWVNVISDLKKIEDLIQSMHIDATLYTESDVHPSCKVTAMKCFLLELQVISLESGDASIHDTVENLIILANNSLSSNGNVTESGCKECEELEEKNIKEFLQSFVHIVQMFINTS

SEQ ID NO: 62 - protein, 578 aa, synthetic construct
  REGION 1..578: note = heavy chian strand (3F815 TL-4)
EVQLQQSGPELVKPGASMKISCKASGYSFTDYIMNWVKQSHGKNLEWIGLSIPYNGGTSYNQKFEGKATLTVDKSSSTAYMELLSLTSEDSAVYYCARGIKGYFAMDYWGQGTSVTVSSASTKGPSVFPLAPSSKSTSGGTAALGCLVKDYFPEPVTVSWNSGALTSGVHTFPAVLQSSGLYSLSSVVTVPSSSLGTQTYICNVNHKPSNTKVDKRVEPKSCDKTHTCPPCPAPELLGGPSVFLFPPKPKDTLMISRTPEVTCVVVDVSHEDPEVKFNWYVDGVEVHNAKTKPREEQYNSTYRVVSVLTVLHQDWLNGKEYKCKVSNKALPAPIEKTISKAKGQPREPQVYTLPPSREEMTKNQVSLTCLVKGFYPSDIAVEWESNGQPENNYKTTPPVLDSDGSFFLYSKLTVDKSRWQQGNVFSCSVMHEALHNHYTQKSLSLSPGKEAAAKEAAAKEAAAKNWVNVISDLKKIEDLIQSMHIDATLYTESDVHPSCKVTAMKCFLLELQVISLESGDASIHDTVENLIILANNSLSSNGNVTESGCKECEELEEKNIKEFLQSFVHIVQMFINTS

SEQ ID NO: 63 - protein, 563 aa, synthetic construct
  REGION 1..563: note = heavy chian strand (3F815 TL-5)
EVQLQQSGPELVKPGASMKISCKASGYSFTDYIMNWVKQSHGKNLEWIGLSIPYNGGTSYNQKFEGKATLTVDKSSSTAYMELLSLTSEDSAVYYCARGIKGYFAMDYWGQGTSVTVSSASTKGPSVFPLAPSSKSTSGGTAALGCLVKDYFPEPVTVSWNSGALTSGVHTFPAVLQSSGLYSLSSVVTVPSSSLGTQTYICNVNHKPSNTKVDKRVEPKSCDKTHTCPPCPAPELLGGPSVFLFPPKPKDTLMISRTPEVTCVVVDVSHEDPEVKFNWYVDGVEVHNAKTKPREEQYNSTYRVVSVLTVLHQDWLNGKEYKCKVSNKALPAPIEKTISKAKGQPREPQVYTLPPSREEMTKNQVSLTCLVKGFYPSDIAVEWESNGQPENNYKTTPPVLDSDGSFFLYSKLTVDKSRWQQGNVFSCSVMHEALHNHYTQKSLSLSPGKNWVNVISDLKKIEDLIQSMHIDATLYTESDVHPSCKVTAMKCFLLELQVISLESGDASIHDTVENLIILANNSLSSNGNVTESGCKECEELEEKNIKEFLQSFVHIVQMFINTS

SEQ ID NO: 64 - protein, 244 aa, synthetic construct
  REGION 1..244: note = hTIGIT
MRWCLLLIWAQGLRQAPLASGMMTGTIETTGNISAEKGGSIILQCHLSSTTAQVTQVNWEQQDQLLAICNADLGWHISPSFKDRVAPGPGLGLTLQSLTVNDTGEYFCIYHTYPDGTYTGRIFLEVLESSVAEHGARFQIPLLGAMAATLVVICTAVIVVVALTRKKKALRIHSVEGDLRRKSAGQEEWSPSAPSPPGSCVQAEAAPAGLCGEQRGEDCAELHDYFNVLSYRSLGNCSFFTETG

SEQ ID NO: 65 - DNA, 354 bp, synthetic construct
  misc_feature 1..354: note = heavy chain variable region coding DNA (7A6)
  source 1..354: mol_type = other DNA
caggtgcagctgcaggagagcggccccggcctggtgaagcccagccagaccctgagcctgacctgcaccgtgaccggctacagcatcaccagcgactacgcctggaactggatcaggcagccccccggcaagggcctggagtggatgggctacatcagctacagcggcagcgccaggtacaaccccagcctgaagagcagggtgaccatcagcagggacaccagcaagaaccagttcagcctgaagctgagcagcgtgaccgccgaggacaccgccacctactactgcgccaggaagggctaccccgcctacttcgcctactggggccagggcaccctggtgaccgtgagcagc

SEQ ID NO: 66 - DNA, 321 bp, synthetic construct
  misc_feature 1..321: note = light chain variable region coding DNA (7A6)
  source 1..321: mol_type = other DNA
gacatccagatgacccagagccccagcagcctgagcgccagcgtgggcgacagggtgagcatcacctgcaaggccagccaggacgtgagcaccgccgtggcctggtaccagcagaagcccggccaggcccccaggctgctgatctacagcgccagctacaggtacaccggcgtgcccgacaggttcagcggcagcggcagcggcaccgacttcaccctgaccatcagcagcctgcagcccgaggacttcgccacctactactgccagcaccactacagcaccccctacaccttcggccagggcaccaagctggagatcaag

SEQ ID NO: 67 - DNA, 990 bp, synthetic construct
  misc_feature 1..990: note = heavy chain constant region coding DNA
  source 1..990: mol_type = other DNA
gccagcaccaagggccccagcgtgttccccctggcccccagcagcaagagcaccagcggcggcaccgccgccctgggctgcctggtgaaggactacttccccgagcccgtgaccgtgagctggaacagcggcgccctgaccagcggcgtgcacaccttccccgccgtgctgcagagcagcggcctgtacagcctgagcagcgtggtgaccgtgcccagcagcagcctgggcacccagacctacatctgcaacgtgaaccacaagcccagcaacaccaaggtggacaagagggtggagcccaagagctgcgacaagacccacacctgccccccctgccccgcccccgagctgctgggcggccccagcgtgttcctgttcccccccaagcccaaggacaccctgatgatcagcaggacccccgaggtgacctgcgtggtggtggacgtgagccacgaggaccccgaggtgaagttcaactggtacgtggacggcgtggaggtgcacaacgccaagaccaagcccagggaggagcagtacaacagcacctacagggtggtgagcgtgctgaccgtgctgcaccaggactggctgaacggcaaggagtacaagtgcaaggtgagcaacaaggccctgcccgcccccatcgagaagaccatcagcaaggccaagggccagcccagggagccccaggtgtacaccctgccccccagcagggaggagatgaccaagaaccaggtgagcctgacctgcctggtgaagggcttctaccccagcgacatcgccgtggagtgggagagcaacggccagcccgagaacaactacaagaccaccccccccgtgctggacagcgacggcagcttcttcctgtacagcaagctgaccgtggacaagagcaggtggcagcagggcaacgtgttcagctgcagcgtgatgcacgaggccctgcacaaccactacacccagaagagcctgagcctgagccccggcaag

SEQ ID NO: 68 - DNA, 321 bp, synthetic construct
  misc_feature 1..321: note = light chain constant region coding DNA
  source 1..321: mol_type = other DNA
aggaccgtggccgcccccagcgtgttcatcttcccccccagcgacgagcagctgaagagcggcaccgccagcgtggtgtgcctgctgaacaacttctaccccagggaggccaaggtgcagtggaaggtggacaacgccctgcagagcggcaacagccaggagagcgtgaccgagcaggacagcaaggacagcacctacagcctgagcagcaccctgaccctgagcaaggccgactacgagaagcacaaggtgtacgcctgcgaggtgacccaccagggcctgagcagccccgtgaccaagagcttcaacaggggcgagtgc

SEQ ID NO: 69 - DNA, 342 bp, synthetic construct
  misc_feature 1..342: note = IL-15 coding DNA
  source 1..342: mol_type = other DNA
aactgggtgaacgtgatcagcgacctgaagaagatcgaggacctgatccagagcatgcacatcgacgccaccctgtacaccgagagcgacgtgcaccccagctgcaaggtgaccgccatgaagtgcttcctgctggagctgcaggtgatcagcctggagagcggcgacgccagcatccacgacaccgtggagaacctgatcatcctggccaacaacagcctgagcagcaacggcaacgtgaccgagagcggctgcaaggagtgcgaggagctggaggagaagaacatcaaggagttcctgcagagcttcgtgcacatcgtgcagatgttcatcaacaccagc

SEQ ID NO: 70 - DNA, 45 bp, synthetic construct
  misc_feature 1..45: note = flexible linker coding DNA
  source 1..45: mol_type = other DNA
ggcggcggcggcagcggcggcggcggcagcggcggcggcggcagc

SEQ ID NO: 71 - DNA, 45 bp, synthetic construct
  misc_feature 1..45: note = rigid linker coding DNA
  source 1..45: mol_type = other DNA
gaggccgccgccaaggaggccgccgccaaggaggccgccgccaag

SEQ ID NO: 72 - DNA, 357 bp, synthetic construct
  misc_feature 1..357: note = heavy chain variable region coding DNA (2B7)
  source 1..357: mol_type = other DNA
gaggtgcagctgcagcagagcggccccgagctggtgaagcccggcgccagcgtgaagatcagctgcaagaccagcggcagcaccttcaccgagtacaccatgcactgggtgaagcagagccacggcaagagcctggagtggatcggcggcctgaaccccaacaacggcggcaccagctacaaccagaggttcaaggacagggccaccctgaccgtggacaagagcagcagcaccgcctacatggagctgaggagcctgaccagcgaggacagcgccgtgtactactgcaccaggggcacctactacgactacagcttcgcctactggggccagggcaccctggtgaccgtgagcgcc

SEQ ID NO: 73 - DNA, 321 bp, synthetic construct
  misc_feature 1..321: note = light chain variable region coding DNA (2B7)
  source 1..321: mol_type = other DNA
gacatcgtgatgacccagagccacaagttcatgagcaccagcgtgggcgacagggtgagcatcacctgcaaggccagccactacgtgagcaccgccgtggcctggtaccagcagaagcccggccagagccccaagctgctgatctacagccccagctacaggtacaccggcgtgcccgacaggttcaccggcagcggcagcggcaccgacttcaccttcaccatcagcagcgtgcaggccgaggacctggccgtgtactactgccaccagcactacagcaccccctggaccttcggcggcggcaccaagctggagatcaag

SEQ ID NO: 74 - DNA, 357 bp, synthetic construct
  misc_feature 1..357: note = heavy chain variable region coding DNA (3F8)
  source 1..357: mol_type = other DNA
gaggtgcagctgcagcagagcggccccgagctggtgaagcccggcgccagcatgaagatcagctgcaaggccagcggctacagcttcaccgactacatcatgaactgggtgaagcagagccacggcaagaacctggagtggatcggcctgagcatcccctacaacggcggcaccagctacaaccagaagttcgagggcaaggccaccctgaccgtggacaagagcagcagcaccgcctacatggagctgctgagcctgaccagcgaggacagcgccgtgtactactgcgccaggggcatcaagggctacttcgccatggactactggggccagggcaccagcgtgaccgtgagcagc

SEQ ID NO: 75 - DNA, 336 bp, synthetic construct
  misc_feature 1..336: note = light chain variable region coding DNA (3F8)
  source 1..336: mol_type = other DNA
gacgtggtggtgacccagacccccctgagcctgcccgtgagcttcggcgaccaggtgagcatcagctgcaggagcagccagagcctggtgaacagcttcggcaagacctacctgagctggttcctgcacaagcccggccagagcccccagctgatcatgtacggcgtgagcaacaggttcagcggcgtgcccgacaggttcagcggcagcggcagcggcaccgacttcaccctgaagatcagcaccatcaagcccgaggacctgggcatgtactactgcctgcagggcacccaccagccctggaccttcggcggcggcaccaagctggagatcaag

SEQ ID NO: 76 - protein, 42 aa, synthetic construct
  REGION 1..42: note = Tag
MAPRRARGCRTLGLPALLLLLLLRPPATRGDYKDDDDKIEGR

SEQ ID NO: 77 - protein, 5 aa, synthetic construct
  REGION 1..5: note = peptide linker
EAAAK

SEQ ID NO: 78 - protein, 7 aa, synthetic construct
  REGION 1..7: note = peptide linker
AEAAAKA

SEQ ID NO: 79 - protein, 12 aa, synthetic construct
  REGION 1..12: note = peptide linker
AEAAAKEAAAKA

SEQ ID NO: 80 - protein, 17 aa, synthetic construct
  REGION 1..17: note = peptide linker
AEAAAKEAAAKEAAAKA

SEQ ID NO: 81 - protein, 22 aa, synthetic construct
  REGION 1..22: note = peptide linker
AEAAAKEAAAKEAAAKEAAAKA

SEQ ID NO: 82 - protein, 27 aa, synthetic construct
  REGION 1..27: note = peptide linker
AEAAAKEAAAKEAAAKEAAAKEAAAKA

SEQ ID NO: 83 - protein, 13 aa, synthetic construct
  REGION 1..13: note = peptide linker
AEAAAKEAAAKAG

SEQ ID NO: 84 - protein, 14 aa, synthetic construct
  REGION 1..14: note = peptide linker
AEAAAKEAAAKAGS

SEQ ID NO: 85 - protein, 5 aa, synthetic construct
  REGION 1..5: note = peptide linker
GGGGG

SEQ ID NO: 86 - protein, 5 aa, synthetic construct
  REGION 1..5: note = peptide linker
GGAGG

SEQ ID NO: 87 - protein, 8 aa, synthetic construct
  REGION 1..8: note = peptide linker
GGGGGGGG

SEQ ID NO: 88 - protein, 10 aa, synthetic construct
  REGION 1..10: note = peptide linker
GAGAGAGAGA

SEQ ID NO: 89 - protein, 18 aa, synthetic construct
  REGION 1..18: note = peptide linker
RPLSYRPPFPFGFPSVRP

SEQ ID NO: 90 - protein, 18 aa, synthetic construct
  REGION 1..18: note = peptide linker
YPRSIYIRRRHPSPSLTT

SEQ ID NO: 91 - protein, 18 aa, synthetic construct
  REGION 1..18: note = peptide linker
TPSHLSHILPSFGLPTFN

SEQ ID NO: 92 - protein, 18 aa, synthetic construct
  REGION 1..18: note = peptide linker
RPVSPFTFPRLSNSWLPA

SEQ ID NO: 93 - protein, 18 aa, synthetic construct
  REGION 1..18: note = peptide linker
SPAAHFPRSIPRPGPIRT

SEQ ID NO: 94 - protein, 18 aa, synthetic construct
  REGION 1..18: note = peptide linker
APGPSAPSHRSLPSRAFG

SEQ ID NO: 95 - protein, 18 aa, synthetic construct
  REGION 1..18: note = peptide linker
PRNSIHFLHPLLVAPLGA

SEQ ID NO: 96 - protein, 18 aa, synthetic construct
  REGION 1..18: note = peptide linker
MPSLSGVLQVRYLSPPDL

SEQ ID NO: 97 - protein, 18 aa, synthetic construct
  REGION 1..18: note = peptide linker
SPQYPSPLTLTLPPHPSL

SEQ ID NO: 98 - protein, 18 aa, synthetic construct
  REGION 1..18: note = peptide linker
NPSLNPPSYLHRAPSRIS

SEQ ID NO: 99 - protein, 17 aa, synthetic construct
  REGION 1..17: note = peptide linker
LPWRTSLLPSLPLRRRP

SEQ ID NO: 100 - protein, 18 aa, synthetic construct
  REGION 1..18: note = peptide linker
PPLFAKGPVGLLSRSFPP

SEQ ID NO: 101 - protein, 18 aa, synthetic construct
  REGION 1..18: note = peptide linker
VPPAPVVSLRSAHARPPY

SEQ ID NO: 102 - protein, 17 aa, synthetic construct
  REGION 1..17: note = peptide linker
LRPTPPRVRSYTCCPTP

SEQ ID NO: 103 - protein, 18 aa, synthetic construct
  REGION 1..18: note = peptide linker
PNVAHVLPLLTVPWDNLR

SEQ ID NO: 104 - protein, 18 aa, synthetic construct
  REGION 1..18: note = peptide linker
CNPLLPLCARSPAVRTFP

SEQ ID NO: 105 - protein, 14 aa, synthetic construct
  REGION 1..14: note = peptide linker
LGTPTPTPTPTGEF

SEQ ID NO: 106 - protein, 8 aa, synthetic construct
  REGION 1..8: note = peptide linker
EDFTRGKL

SEQ ID NO: 107 - protein, 21 aa, synthetic construct
  REGION 1..21: note = peptide linker
LEAAAREAAAREAAAREAAAR

SEQ ID NO: 108 - protein, 16 aa, synthetic construct
  REGION 1..16: note = peptide linker
LEAAAREAAAREAAAR

SEQ ID NO: 109 - protein, 6 aa, synthetic construct
  REGION 1..6: note = peptide linker
LEAAAR

SEQ ID NO: 110 - protein, 11 aa, synthetic construct
  REGION 1..11: note = peptide linker
LEAAAREAAAR

SEQ ID NO: 111 - protein, 20 aa, synthetic construct
  REGION 1..20: note = peptide linker
EAAAREAAAREAAAREAAAR

SEQ ID NO: 112 - protein, 15 aa, synthetic construct
  REGION 1..15: note = peptide linker
EAAAREAAAREAAAR

SEQ ID NO: 113 - protein, 10 aa, synthetic construct
  REGION 1..10: note = peptide linker
EAAAREAAAR

SEQ ID NO: 114 - protein, 5 aa, synthetic construct
  REGION 1..5: note = peptide linker
EAAAR

SEQ ID NO: 115 - protein, 10 aa, synthetic construct
  REGION 1..10: note = peptide linker
LTEEQQEGGG

SEQ ID NO: 116 - protein, 9 aa, synthetic construct
  REGION 1..9: note = peptide linker
TEEQQEGGG

SEQ ID NO: 117 - protein, 19 aa, synthetic construct
  REGION 1..19: note = peptide linker
LAKLKQKTEQLQDRIAGGG

SEQ ID NO: 118 - protein, 10 aa, synthetic construct
  REGION 1..10: note = peptide linker
LELKTPLGDT

SEQ ID NO: 119 - protein, 10 aa, synthetic construct
  REGION 1..10: note = peptide linker
THTCPRCPEP

SEQ ID NO: 120 - protein, 10 aa, synthetic construct
  REGION 1..10: note = peptide linker
KSCDTPPPCP

SEQ ID NO: 121 - protein, 10 aa, synthetic construct
  REGION 1..10: note = peptide linker
RCPEPKSCDT

SEQ ID NO: 122 - protein, 10 aa, synthetic construct
  REGION 1..10: note = peptide linker
PPPCPRCPEP

SEQ ID NO: 123 - protein, 10 aa, synthetic construct
  REGION 1..10: note = peptide linker
KSCDTPPPCP

SEQ ID NO: 124 - protein, 5 aa, synthetic construct
  REGION 1..5: note = peptide linker
RCPGG

SEQ ID NO: 125 - protein, 18 aa, synthetic construct
  REGION 1..18: note = peptide linker
LEPKSSDKTHTSPPSPGG